European Patent Application EP 4 299 803 A2, published January 3, 2024. Title: MACROMOLECULE ANALYSIS EMPLOYING NUCLEIC ACID ENCODING. Applicant: Encodia, Inc. Application EP. The sequence listing filed with the application follows.

SEQUENCE LISTING (188 sequences)

SEQ ID NO: 1 - DNA, 15 bp, synthetic construct
  misc_feature 1..15: note = oligonucleotide barcode BC_1
  source 1..15: mol_type = other DNA
atgtctagcatgccg

SEQ ID NO: 2 - DNA, 15 bp, synthetic construct
  misc_feature 1..15: note = oligonucleotide barcode BC_2
  source 1..15: mol_type = other DNA
ccgtgtcatgtggaa

SEQ ID NO: 3 - DNA, 15 bp, synthetic construct
  misc_feature 1..15: note = oligonucleotide barcode BC_3
  source 1..15: mol_type = other DNA
taagccggtatatca

SEQ ID NO: 4 - DNA, 15 bp, synthetic construct
  misc_feature 1..15: note = oligonucleotide barcode BC_4
  source 1..15: mol_type = other DNA
ttcgatatgacggaa

SEQ ID NO: 5 - DNA, 15 bp, synthetic construct
  misc_feature 1..15: note = oligonucleotide barcode BC_5
  source 1..15: mol_type = other DNA
cgtatacgcgttagg

SEQ ID NO: 6 - DNA, 15 bp, synthetic construct
  misc_feature 1..15: note = oligonucleotide barcode BC_6
  source 1..15: mol_type = other DNA
aactgccgagattcc

SEQ ID NO: 7 - DNA, 15 bp, synthetic construct
  misc_feature 1..15: note = oligonucleotide barcode BC_7
  source 1..15: mol_type = other DNA
tgatcttagctgtgc

SEQ ID NO: 8 - DNA, 15 bp, synthetic construct
  misc_feature 1..15: note = oligonucleotide barcode BC_8
  source 1..15: mol_type = other DNA
gagtcggtaccttga

SEQ ID NO: 9 - DNA, 15 bp, synthetic construct
  misc_feature 1..15: note = oligonucleotide barcode BC_9
  source 1..15: mol_type = other DNA
ccgcttgtgatctgg

SEQ ID NO: 10 - DNA, 15 bp, synthetic construct
  misc_feature 1..15: note = oligonucleotide barcode BC_10
  source 1..15: mol_type = other DNA
agatagcgtaccgga

SEQ ID NO: 11 - DNA, 15 bp, synthetic construct
  misc_feature 1..15: note = oligonucleotide barcode BC_11
  source 1..15: mol_type = other DNA
tccaggctcatcatc

SEQ ID NO: 12 - DNA, 15 bp, synthetic construct
  misc_feature 1..15: note = oligonucleotide barcode BC_12
  source 1..15: mol_type = other DNA
gagtactagagccaa

SEQ ID NO: 13 - DNA, 15 bp, synthetic construct
  misc_feature 1..15: note = oligonucleotide barcode BC_13
  source 1..15: mol_type = other DNA
gagcgtcaataacgg

SEQ ID NO: 14 - DNA, 15 bp, synthetic construct
  misc_feature 1..15: note = oligonucleotide barcode BC_14
  source 1..15: mol_type = other DNA
gcggtatctacactg

SEQ ID NO: 15 - DNA, 15 bp, synthetic construct
  misc_feature 1..15: note = oligonucleotide barcode BC_15
  source 1..15: mol_type = other DNA
cttctccgaagagaa

SEQ ID NO: 16 - DNA, 15 bp, synthetic construct
  misc_feature 1..15: note = oligonucleotide barcode BC_16
  source 1..15: mol_type = other DNA
tgaagcctgtgttaa

SEQ ID NO: 17 - DNA, 15 bp, synthetic construct
  misc_feature 1..15: note = oligonucleotide barcode BC_17
  source 1..15: mol_type = other DNA
ctggatggttgtcga

SEQ ID NO: 18 - DNA, 15 bp, synthetic construct
  misc_feature 1..15: note = oligonucleotide barcode BC_18
  source 1..15: mol_type = other DNA
actgcacggttccaa

SEQ ID NO: 19 - DNA, 15 bp, synthetic construct
  misc_feature 1..15: note = oligonucleotide barcode BC_19
  source 1..15: mol_type = other DNA
cgagagatggtcctt

SEQ ID NO: 20 - DNA, 15 bp, synthetic construct
  misc_feature 1..15: note = oligonucleotide barcode BC_20
  source 1..15: mol_type = other DNA
tcttgagagacaaga

SEQ ID NO: 21 - DNA, 15 bp, synthetic construct
  misc_feature 1..15: note = oligonucleotide barcode BC_21
  source 1..15: mol_type = other DNA
aattcgcactgtgtt

SEQ ID NO: 22 - DNA, 15 bp, synthetic construct
  misc_feature 1..15: note = oligonucleotide barcode BC_22
  source 1..15: mol_type = other DNA
gtagtgccgctaaga

SEQ ID NO: 23 - DNA, 15 bp, synthetic construct
  misc_feature 1..15: note = oligonucleotide barcode BC_23
  source 1..15: mol_type = other DNA
cctatagcacaatcc

SEQ ID NO: 24 - DNA, 15 bp, synthetic construct
  misc_feature 1..15: note = oligonucleotide barcode BC_24
  source 1..15: mol_type = other DNA
atcaccgaggttgga

SEQ ID NO: 25 - DNA, 15 bp, synthetic construct
  misc_feature 1..15: note = oligonucleotide barcode BC_25
  source 1..15: mol_type = other DNA
gattcaacggagaag

SEQ ID NO: 26 - DNA, 15 bp, synthetic construct
  misc_feature 1..15: note = oligonucleotide barcode BC_26
  source 1..15: mol_type = other DNA
acgaacctcgcacca

SEQ ID NO: 27 - DNA, 15 bp, synthetic construct
  misc_feature 1..15: note = oligonucleotide barcode BC_27
  source 1..15: mol_type = other DNA
aggacttcaagaaga

SEQ ID NO: 28 - DNA, 15 bp, synthetic construct
  misc_feature 1..15: note = oligonucleotide barcode BC_28
  source 1..15: mol_type = other DNA
ggttgaatcctcgca

SEQ ID NO: 29 - DNA, 15 bp, synthetic construct
  misc_feature 1..15: note = oligonucleotide barcode BC_29
  source 1..15: mol_type = other DNA
aaccaacctctagcg

SEQ ID NO: 30 - DNA, 15 bp, synthetic construct
  misc_feature 1..15: note = oligonucleotide barcode BC_30
  source 1..15: mol_type = other DNA
acgcgaatatctaac

SEQ ID NO: 31 - DNA, 15 bp, synthetic construct
  misc_feature 1..15: note = oligonucleotide barcode BC_31
  source 1..15: mol_type = other DNA
gttgagaattacacc

SEQ ID NO: 32 - DNA, 15 bp, synthetic construct
  misc_feature 1..15: note = oligonucleotide barcode BC_32
  source 1..15: mol_type = other DNA
ctctctctgtgaacc

SEQ ID NO: 33 - DNA, 15 bp, synthetic construct
  misc_feature 1..15: note = oligonucleotide barcode BC_33
  source 1..15: mol_type = other DNA
gccatcagtaagaga

SEQ ID NO: 34 - DNA, 15 bp, synthetic construct
  misc_feature 1..15: note = oligonucleotide barcode BC_34
  source 1..15: mol_type = other DNA
gcaacgtgaattgag

SEQ ID NO: 35 - DNA, 15 bp, synthetic construct
  misc_feature 1..15: note = oligonucleotide barcode BC_35
  source 1..15: mol_type = other DNA
ctaagtagagccaca

SEQ ID NO: 36 - DNA, 15 bp, synthetic construct
  misc_feature 1..15: note = oligonucleotide barcode BC_36
  source 1..15: mol_type = other DNA
tgtctgttggaagcg

SEQ ID NO: 37 - DNA, 15 bp, synthetic construct
  misc_feature 1..15: note = oligonucleotide barcode BC_37
  source 1..15: mol_type = other DNA
ttaatagacagcgcg

SEQ ID NO: 38 - DNA, 15 bp, synthetic construct
  misc_feature 1..15: note = oligonucleotide barcode BC_38
  source 1..15: mol_type = other DNA
cgacgctctaacaag

SEQ ID NO: 39 - DNA, 15 bp, synthetic construct
  misc_feature 1..15: note = oligonucleotide barcode BC_39
  source 1..15: mol_type = other DNA
catggcttattgaga

SEQ ID NO: 40 - DNA, 15 bp, synthetic construct
  misc_feature 1..15: note = oligonucleotide barcode BC_40
  source 1..15: mol_type = other DNA
actaggtatggccgg

SEQ ID NO: 41 - DNA, 15 bp, synthetic construct
  misc_feature 1..15: note = oligonucleotide barcode BC_41
  source 1..15: mol_type = other DNA
gtcctcgtctatcct

SEQ ID NO: 42 - DNA, 15 bp, synthetic construct
  misc_feature 1..15: note = oligonucleotide barcode BC_42
  source 1..15: mol_type = other DNA
taggattccgttacc

SEQ ID NO: 43 - DNA, 15 bp, synthetic construct
  misc_feature 1..15: note = oligonucleotide barcode BC_43
  source 1..15: mol_type = other DNA
tctgaccaccggaag

SEQ ID NO: 44 - DNA, 15 bp, synthetic construct
  misc_feature 1..15: note = oligonucleotide barcode BC_44
  source 1..15: mol_type = other DNA
agagtcacctcgtgg

SEQ ID NO: 45 - DNA, 15 bp, synthetic construct
  misc_feature 1..15: note = oligonucleotide barcode BC_45
  source 1..15: mol_type = other DNA
ctgatgtagtcgaag

SEQ ID NO: 46 - DNA, 15 bp, synthetic construct
  misc_feature 1..15: note = oligonucleotide barcode BC_46
  source 1..15: mol_type = other DNA
gtcggttgcggatag

SEQ ID NO: 47 - DNA, 15 bp, synthetic construct
  misc_feature 1..15: note = oligonucleotide barcode BC_47
  source 1..15: mol_type = other DNA
tcctcctcctaagaa

SEQ ID NO: 48 - DNA, 15 bp, synthetic construct
  misc_feature 1..15: note = oligonucleotide barcode BC_48
  source 1..15: mol_type = other DNA
attcggtccacttca

SEQ ID NO: 49 - DNA, 15 bp, synthetic construct
  misc_feature 1..15: note = oligonucleotide barcode BC_49
  source 1..15: mol_type = other DNA
ccttacaggtctgcg

SEQ ID NO: 50 - DNA, 15 bp, synthetic construct
  misc_feature 1..15: note = oligonucleotide barcode BC_50
  source 1..15: mol_type = other DNA
gatcattggccaatt

SEQ ID NO: 51 - DNA, 15 bp, synthetic construct
  misc_feature 1..15: note = oligonucleotide barcode BC_51
  source 1..15: mol_type = other DNA
ttcaaggctgagttg

SEQ ID NO: 52 - DNA, 15 bp, synthetic construct
  misc_feature 1..15: note = oligonucleotide barcode BC_52
  source 1..15: mol_type = other DNA
tggctcgattgaatc

SEQ ID NO: 53 - DNA, 15 bp, synthetic construct
  misc_feature 1..15: note = oligonucleotide barcode BC_53
  source 1..15: mol_type = other DNA
gtaagccatccgctc

SEQ ID NO: 54 - DNA, 15 bp, synthetic construct
  misc_feature 1..15: note = oligonucleotide barcode BC_54
  source 1..15: mol_type = other DNA
acacatgcgtagaca

SEQ ID NO: 55 - DNA, 15 bp, synthetic construct
  misc_feature 1..15: note = oligonucleotide barcode BC_55
  source 1..15: mol_type = other DNA
tgctatggattcaag

SEQ ID NO: 56 - DNA, 15 bp, synthetic construct
  misc_feature 1..15: note = oligonucleotide barcode BC_56
  source 1..15: mol_type = other DNA
ccacgaggcttagtt

SEQ ID NO: 57 - DNA, 15 bp, synthetic construct
  misc_feature 1..15: note = oligonucleotide barcode BC_57
  source 1..15: mol_type = other DNA
ggccaactaaggtgc

SEQ ID NO: 58 - DNA, 15 bp, synthetic construct
  misc_feature 1..15: note = oligonucleotide barcode BC_58
  source 1..15: mol_type = other DNA
gcacctattcgacaa

SEQ ID NO: 59 - DNA, 15 bp, synthetic construct
  misc_feature 1..15: note = oligonucleotide barcode BC_59
  source 1..15: mol_type = other DNA
tggacacgatcggct

SEQ ID NO: 60 - DNA, 15 bp, synthetic construct
  misc_feature 1..15: note = oligonucleotide barcode BC_60
  source 1..15: mol_type = other DNA
ctataattccaacgg

SEQ ID NO: 61 - DNA, 15 bp, synthetic construct
  misc_feature 1..15: note = oligonucleotide barcode BC_61
  source 1..15: mol_type = other DNA
aacgtggttagtaag

SEQ ID NO: 62 - DNA, 15 bp, synthetic construct
  misc_feature 1..15: note = oligonucleotide barcode BC_62
  source 1..15: mol_type = other DNA
caaggaacgagtggc

SEQ ID NO: 63 - DNA, 15 bp, synthetic construct
  misc_feature 1..15: note = oligonucleotide barcode BC_63
  source 1..15: mol_type = other DNA
caccagaacggaaga

SEQ ID NO: 64 - DNA, 15 bp, synthetic construct
  misc_feature 1..15: note = oligonucleotide barcode BC_64
  source 1..15: mol_type = other DNA
cgtacggtcaagcaa

SEQ ID NO: 65 - DNA, 15 bp, synthetic construct
  misc_feature 1..15: note = oligonucleotide barcode BC_65
  source 1..15: mol_type = other DNA
tcggtgacaggctaa

SEQ ID NO: 66 - DNA, 15 bp, synthetic construct
  misc_feature 1..15: note = oligonucleotide barcode BC_1 REV
  source 1..15: mol_type = other DNA
cggcatgctagacat

SEQ ID NO: 67 - DNA, 15 bp, synthetic construct
  misc_feature 1..15: note = oligonucleotide barcode BC_2REV
  source 1..15: mol_type = other DNA
ttccacatgacacgg

SEQ ID NO: 68 - DNA, 15 bp, synthetic construct
  misc_feature 1..15: note = oligonucleotide barcode BC_3REV
  source 1..15: mol_type = other DNA
tgatataccggctta

SEQ ID NO: 69 - DNA, 15 bp, synthetic construct
  misc_feature 1..15: note = oligonucleotide barcode BC_4REV
  source 1..15: mol_type = other DNA
ttccgtcatatcgaa

SEQ ID NO: 70 - DNA, 15 bp, synthetic construct
  misc_feature 1..15: note = oligonucleotide barcode BC_5REV
  source 1..15: mol_type = other DNA
cctaacgcgtatacg

SEQ ID NO: 71 - DNA, 15 bp, synthetic construct
  misc_feature 1..15: note = oligonucleotide barcode BC_6REV
  source 1..15: mol_type = other DNA
ggaatctcggcagtt

SEQ ID NO: 72 - DNA, 15 bp, synthetic construct
  misc_feature 1..15: note = oligonucleotide barcode BC_7REV
  source 1..15: mol_type = other DNA
gcacagctaagatca

SEQ ID NO: 73 - DNA, 15 bp, synthetic construct
  misc_feature 1..15: note = oligonucleotide barcode BC_8REV
  source 1..15: mol_type = other DNA
tcaaggtaccgactc

SEQ ID NO: 74 - DNA, 15 bp, synthetic construct
  misc_feature 1..15: note = oligonucleotide barcode BC_9REV
  source 1..15: mol_type = other DNA
ccagatcacaagcgg

SEQ ID NO: 75 - DNA, 15 bp, synthetic construct
  misc_feature 1..15: note = oligonucleotide barcode BC_10REV
  source 1..15: mol_type = other DNA
tccggtacgctatct

SEQ ID NO: 76 - DNA, 15 bp, synthetic construct
  misc_feature 1..15: note = oligonucleotide barcode BC_11REV
  source 1..15: mol_type = other DNA
gatgatgagcctgga

SEQ ID NO: 77 - DNA, 15 bp, synthetic construct
  misc_feature 1..15: note = oligonucleotide barcode BC_12REV
  source 1..15: mol_type = other DNA
ttggctctagtactc

SEQ ID NO: 78 - DNA, 15 bp, synthetic construct
  misc_feature 1..15: note = oligonucleotide barcode BC_13REV
  source 1..15: mol_type = other DNA
ccgttattgacgctc

SEQ ID NO: 79 - DNA, 15 bp, synthetic construct
  misc_feature 1..15: note = oligonucleotide barcode BC_14REV
  source 1..15: mol_type = other DNA
cagtgtagataccgc

SEQ ID NO: 80 - DNA, 15 bp, synthetic construct
  misc_feature 1..15: note = oligonucleotide barcode BC_15REV
  source 1..15: mol_type = other DNA
ttctcttcggagaag

SEQ ID NO: 81 - DNA, 15 bp, synthetic construct
  misc_feature 1..15: note = oligonucleotide barcode BC_16REV
  source 1..15: mol_type = other DNA
ttaacacaggcttca

SEQ ID NO: 82 - DNA, 15 bp, synthetic construct
  misc_feature 1..15: note = oligonucleotide barcode BC_17REV
  source 1..15: mol_type = other DNA
tcgacaaccatccag

SEQ ID NO: 83 - DNA, 15 bp, synthetic construct
  misc_feature 1..15: note = oligonucleotide barcode BC_18REV
  source 1..15: mol_type = other DNA
ttggaaccgtgcagt

SEQ ID NO: 84 - DNA, 15 bp, synthetic construct
  misc_feature 1..15: note = oligonucleotide barcode BC_19 REV
  source 1..15: mol_type = other DNA
aaggaccatctctcg

SEQ ID NO: 85 - DNA, 15 bp, synthetic construct
  misc_feature 1..15: note = oligonucleotide barcode BC_20 REV
  source 1..15: mol_type = other DNA
tcttgtctctcaaga

SEQ ID NO: 86 - DNA, 15 bp, synthetic construct
  misc_feature 1..15: note = oligonucleotide barcode BC_21 REV
  source 1..15: mol_type = other DNA
aacacagtgcgaatt

SEQ ID NO: 87 - DNA, 15 bp, synthetic construct
  misc_feature 1..15: note = oligonucleotide barcode BC_22 REV
  source 1..15: mol_type = other DNA
tcttagcggcactac

SEQ ID NO: 88 - DNA, 15 bp, synthetic construct
  misc_feature 1..15: note = oligonucleotide barcode BC_23 REV
  source 1..15: mol_type = other DNA
ggattgtgctatagg

SEQ ID NO: 89 - DNA, 15 bp, synthetic construct
  misc_feature 1..15: note = oligonucleotide barcode BC_24 REV
  source 1..15: mol_type = other DNA
tccaacctcggtgat

SEQ ID NO: 90 - DNA, 15 bp, synthetic construct
  misc_feature 1..15: note = oligonucleotide barcode BC_25 REV
  source 1..15: mol_type = other DNA
cttctccgttgaatc

SEQ ID NO: 91 - DNA, 15 bp, synthetic construct
  source 1..15: mol_type = other DNA
  misc_feature 1..15: note = oligonucleotide barcode BC_26 REV
tggtgcgaggttcgt

SEQ ID NO: 92 - DNA, 15 bp, synthetic construct
  misc_feature 1..15: note = oligonucleotide barcode BC_27 REV
  source 1..15: mol_type = other DNA
tcttcttgaagtcct

SEQ ID NO: 93 - DNA, 15 bp, synthetic construct
  misc_feature 1..15: note = oligonucleotide barcode BC_28 REV
  source 1..15: mol_type = other DNA
tgcgaggattcaacc

SEQ ID NO: 94 - DNA, 15 bp, synthetic construct
  misc_feature 1..15: note = oligonucleotide barcode BC_29 REV
  source 1..15: mol_type = other DNA
cgctagaggttggtt

SEQ ID NO: 95 - DNA, 15 bp, synthetic construct
  misc_feature 1..15: note = oligonucleotide barcode BC_30 REV
  source 1..15: mol_type = other DNA
gttagatattcgcgt

SEQ ID NO: 96 - DNA, 15 bp, synthetic construct
  misc_feature 1..15: note = oligonucleotide barcode BC_31 REV
  source 1..15: mol_type = other DNA
ggtgtaattctcaac

SEQ ID NO: 97 - DNA, 15 bp, synthetic construct
  misc_feature 1..15: note = oligonucleotide barcode BC_32 REV
  source 1..15: mol_type = other DNA
ggttcacagagagag

SEQ ID NO: 98 - DNA, 15 bp, synthetic construct
  misc_feature 1..15: note = oligonucleotide barcode BC_33 REV
  source 1..15: mol_type = other DNA
tctcttactgatggc

SEQ ID NO: 99 - DNA, 15 bp, synthetic construct
  misc_feature 1..15: note = oligonucleotide barcode BC_34 REV
  source 1..15: mol_type = other DNA
ctcaattcacgttgc

SEQ ID NO: 100 - DNA, 15 bp, synthetic construct
  misc_feature 1..15: note = oligonucleotide barcode BC_35 REV
  source 1..15: mol_type = other DNA
tgtggctctacttag

SEQ ID NO: 101 - DNA, 15 bp, synthetic construct
  misc_feature 1..15: note = oligonucleotide barcode BC_36 REV
  source 1..15: mol_type = other DNA
cgcttccaacagaca

SEQ ID NO: 102 - DNA, 15 bp, synthetic construct
  misc_feature 1..15: note = oligonucleotide barcode BC_37 REV
  source 1..15: mol_type = other DNA
cgcgctgtctattaa

SEQ ID NO: 103 - DNA, 15 bp, synthetic construct
  misc_feature 1..15: note = oligonucleotide barcode BC_38 REV
  source 1..15: mol_type = other DNA
cttgttagagcgtcg

SEQ ID NO: 104 - DNA, 15 bp, synthetic construct
  misc_feature 1..15: note = oligonucleotide barcode BC_39 REV
  source 1..15: mol_type = other DNA
tctcaataagccatg

SEQ ID NO: 105 - DNA, 15 bp, synthetic construct
  misc_feature 1..15: note = oligonucleotide barcode BC_40 REV
  source 1..15: mol_type = other DNA
ccggccatacctagt

SEQ ID NO: 106 - DNA, 15 bp, synthetic construct
  misc_feature 1..15: note = oligonucleotide barcode BC_41 REV
  source 1..15: mol_type = other DNA
aggatagacgaggac

SEQ ID NO: 107 - DNA, 15 bp, synthetic construct
  misc_feature 1..15: note = oligonucleotide barcode BC_42 REV
  source 1..15: mol_type = other DNA
ggtaacggaatccta

SEQ ID NO: 108 - DNA, 15 bp, synthetic construct
  misc_feature 1..15: note = oligonucleotide barcode BC_43 REV
  source 1..15: mol_type = other DNA
cttccggtggtcaga

SEQ ID NO: 109 - DNA, 15 bp, synthetic construct
  misc_feature 1..15: note = oligonucleotide barcode BC_44 REV
  source 1..15: mol_type = other DNA
ccacgaggtgactct

SEQ ID NO: 110 - DNA, 15 bp, synthetic construct
  misc_feature 1..15: note = oligonucleotide barcode BC_45 REV
  source 1..15: mol_type = other DNA
cttcgactacatcag

SEQ ID NO: 111 - DNA, 15 bp, synthetic construct
  misc_feature 1..15: note = oligonucleotide barcode BC_46 REV
  source 1..15: mol_type = other DNA
ctatccgcaaccgac

SEQ ID NO: 112 - DNA, 15 bp, synthetic construct
  misc_feature 1..15: note = oligonucleotide barcode BC_47 REV
  source 1..15: mol_type = other DNA
ttcttaggaggagga

SEQ ID NO: 113 - DNA, 15 bp, synthetic construct
  misc_feature 1..15: note = oligonucleotide barcode BC_48 REV
  source 1..15: mol_type = other DNA
tgaagtggaccgaat

SEQ ID NO: 114 - DNA, 15 bp, synthetic construct
  misc_feature 1..15: note = oligonucleotide barcode BC_49 REV
  source 1..15: mol_type = other DNA
cgcagacctgtaagg

SEQ ID NO: 115 - DNA, 15 bp, synthetic construct
  misc_feature 1..15: note = oligonucleotide barcode BC_50 REV
  source 1..15: mol_type = other DNA
aattggccaatgatc

SEQ ID NO: 116 - DNA, 15 bp, synthetic construct
  misc_feature 1..15: note = oligonucleotide barcode BC_51 REV
  source 1..15: mol_type = other DNA
caactcagccttgaa

SEQ ID NO: 117 - DNA, 15 bp, synthetic construct
  misc_feature 1..15: note = oligonucleotide barcode BC_52 REV
  source 1..15: mol_type = other DNA
gattcaatcgagcca

SEQ ID NO: 118 - DNA, 15 bp, synthetic construct
  misc_feature 1..15: note = oligonucleotide barcode BC_53 REV
  source 1..15: mol_type = other DNA
gagcggatggcttac

SEQ ID NO: 119 - DNA, 15 bp, synthetic construct
  misc_feature 1..15: note = oligonucleotide barcode BC_54 REV
  source 1..15: mol_type = other DNA
tgtctacgcatgtgt

SEQ ID NO: 120 - DNA, 15 bp, synthetic construct
  misc_feature 1..15: note = oligonucleotide barcode BC_55 REV
  source 1..15: mol_type = other DNA
cttgaatccatagca

SEQ ID NO: 121 - DNA, 15 bp, synthetic construct
  misc_feature 1..15: note = oligonucleotide barcode BC_56 REV
  source 1..15: mol_type = other DNA
aactaagcctcgtgg

SEQ ID NO: 122 - DNA, 15 bp, synthetic construct
  misc_feature 1..15: note = oligonucleotide barcode BC_57 REV
  source 1..15: mol_type = other DNA
gcaccttagttggcc

SEQ ID NO: 123 - DNA, 15 bp, synthetic construct
  misc_feature 1..15: note = oligonucleotide barcode BC_58 REV
  source 1..15: mol_type = other DNA
ttgtcgaataggtgc

SEQ ID NO: 124 - DNA, 15 bp, synthetic construct
  misc_feature 1..15: note = oligonucleotide barcode BC_59 REV
  source 1..15: mol_type = other DNA
agccgatcgtgtcca

SEQ ID NO: 125 - DNA, 15 bp, synthetic construct
  misc_feature 1..15: note = oligonucleotide barcode BC_60 REV
  source 1..15: mol_type = other DNA
ccgttggaattatag

SEQ ID NO: 126 - DNA, 15 bp, synthetic construct
  misc_feature 1..15: note = oligonucleotide barcode BC_61 REV
  source 1..15: mol_type = other DNA
cttactaaccacgtt

SEQ ID NO: 127 - DNA, 15 bp, synthetic construct
  misc_feature 1..15: note = oligonucleotide barcode BC_62 REV
  source 1..15: mol_type = other DNA
gccactcgttccttg

SEQ ID NO: 128 - DNA, 15 bp, synthetic construct
  misc_feature 1..15: note = oligonucleotide barcode BC_63 REV
  source 1..15: mol_type = other DNA
tcttccgttctggtg

SEQ ID NO: 129 - DNA, 15 bp, synthetic construct
  misc_feature 1..15: note = oligonucleotide barcode BC_64 REV
  source 1..15: mol_type = other DNA
ttgcttgaccgtacg

SEQ ID NO: 130 - DNA, 15 bp, synthetic construct
  misc_feature 1..15: note = oligonucleotide barcode BC_65 REV
  source 1..15: mol_type = other DNA
ttagcctgtcaccga

SEQ ID NO: 131 - protein, 16 aa, synthetic construct
  REGION 1..16: note = synthetic peptide
  MOD_RES 1: note = formyl-Methionine
MDVEAWLGARVPLVET

SEQ ID NO: 132 - protein, 10 aa, synthetic construct
  REGION 1..10: note = synthetic peptide
TENLYFQNHV

SEQ ID NO: 133 - DNA, 20 bp, synthetic construct
  misc_feature 1..20: note = oligonucleotide primer
  source 1..20: mol_type = other DNA
aatgatacggcgaccaccga

SEQ ID NO: 134 - DNA, 24 bp, synthetic construct
  misc_feature 1..24: note = oligonucleotide primer
  source 1..24: mol_type = other DNA
caagcagaagacggcatacgagat

SEQ ID NO: 135 - skipped

SEQ ID NO: 136 - protein, 8 aa, synthetic construct
  REGION 1..8: note = synthetic peptide
DYKDDDDK

SEQ ID NO: 137 - protein, 14 aa, synthetic construct
  REGION 1..14: note = synthetic peptide
GKPIPNPLLGLDST

SEQ ID NO: 138 - protein, 10 aa, synthetic construct
  REGION 1..10: note = synthetic peptide
EQKLISEEDL

SEQ ID NO: 139 - protein, 9 aa, synthetic construct
  REGION 1..9: note = synthetic peptide
YPYDVPDYA

SEQ ID NO: 140 - protein, 9 aa, synthetic construct
  REGION 1..9: note = synthetic peptide
NWSHPQFEK

SEQ ID NO: 141 - DNA, 82 bp, synthetic construct
  misc_feature 1..82: note = synthetic oligonucleotide
  source 1..82: mol_type = other DNA
tttttgcaaatggcattctgacatcccgtagtccgcgacactagatgtctagcatgccgccgtgtcatgtggaaactgagtg

SEQ ID NO: 142 - DNA, 72 bp, synthetic construct
  misc_feature 1..72: note = synthetic oligonucleotide
  source 1..72: mol_type = other DNA
ttttttttttgactggttccaattgacaagccgtagtccgcgacactagtaagccggtatatcaactgagtg

SEQ ID NO: 143 - DNA, 10 bp, synthetic construct
  misc_feature 1..10: note = synthetic oligonucleotide
  misc_feature 10: note = three carbon (3C) spacer
  source 1..10: mol_type = other DNA
tttttttttt

SEQ ID NO: 144 - DNA, 31 bp, synthetic construct
  misc_feature 1..31: note = synthetic oligonucleotide
  misc_feature 31: note = 18-atom hexa-ethyleneglycol spacer
  source 1..31: mol_type = other DNA
ggatgtcagaatgccatttgctttttttttt

SEQ ID NO: 145 - DNA, 31 bp, synthetic construct; identical to SEQ ID NO: 144
  misc_feature 1..31: note = synthetic oligonucleotide
  misc_feature 31: note = 18-atom hexa-ethyleneglycol spacer
  source 1..31: mol_type = other DNA

SEQ ID NO: 146 - DNA, 31 bp, synthetic construct; identical to SEQ ID NO: 144
  misc_feature 1..31: note = synthetic oligonucleotide
  misc_feature 31: note = five 18-atom hexa-ethyleneglycol spacer
  source 1..31: mol_type = other DNA

SEQ ID NO: 147 - DNA, 25 bp, synthetic construct
  misc_feature 1..25: note = synthetic oligonucleotide
  misc_feature 25: note = 18-atom hexa-ethyleneglycol spacer
  source 1..25: mol_type = other DNA
gcttgtcaattggaaccagtctttt

SEQ ID NO: 148 - DNA, 44 bp, synthetic construct
  misc_feature 1..44: note = synthetic oligonucleotide
  misc_feature 44: note = three carbon (3C) spacer
  source 1..44: mol_type = other DNA
cgatttgcaaggatcactcgtcactcagtcctaacgcgtatacg

SEQ ID NO: 149-150 - skipped (2 entries)

SEQ ID NO: 151 - DNA, 18 bp, synthetic construct
  misc_feature 1..18: note = oligonucleotide primer
  source 1..18: mol_type = other DNA
cgtagtccgcgacactag

SEQ ID NO: 152 - DNA, 20 bp, synthetic construct
  misc_feature 1..20: note = oligonucleotide primer
  source 1..20: mol_type = other DNA
cgatttgcaaggatcactcg

SEQ ID NO: 153 - DNA, 21 bp, synthetic construct
  misc_feature 1..21: note = synthetic oligonucleotide
  source 1..21: mol_type = other DNA
gcaaatggcattctgacatcc

SEQ ID NO: 154 - DNA, 21 bp, synthetic construct
  misc_feature 1..21: note = synthetic oligonucleotide
  source 1..21: mol_type = other DNA
gactggttccaattgacaagc

SEQ ID NO: 155 - DNA, 23 bp, synthetic construct
  misc_feature 1..23: note = synthetic oligonucleotide
  misc_feature 23: note = three carbon (3C) spacer
  source 1..23: mol_type = other DNA
cgtatacgcgttaggactgagtg

SEQ ID NO: 156 - DNA, 38 bp, synthetic construct
  misc_feature 1..38: note = synthetic oligonucleotide
  misc_feature 38: note = three carbon (3C) spacer
  source 1..38: mol_type = other DNA
aactgccgagattcccgtatacgcgttaggactgagtg

SEQ ID NO: 157 - DNA, 46 bp, synthetic construct
  misc_feature 1..46: note = oligonucleotide primer
  source 1..46: mol_type = other DNA
agtccgcgcaatcagatgtctagcatgccggatccggatcgatctc

SEQ ID NO: 158 - DNA, 46 bp, synthetic construct
  misc_feature 1..46: note = oligonucleotide primer
  source 1..46: mol_type = other DNA
agtccgcgcaatcagccgtgtcatgtggaagatccggatcgatctc

SEQ ID NO: 159 - DNA, 46 bp, synthetic construct
  misc_feature 1..46: note = oligonucleotide primer
  source 1..46: mol_type = other DNA
agtccgcgcaatcagtaagccggtatatcagatccggatcgatctc

SEQ ID NO: 160 - DNA, 46 bp, synthetic construct
  misc_feature 1..46: note = oligonucleotide primer
  source 1..46: mol_type = other DNA
agtccgcgcaatcagttcgatatgacggaagatccggatcgatctc

SEQ ID NO: 161 - DNA, 46 bp, synthetic construct
  misc_feature 1..46: note = oligonucleotide primer
  source 1..46: mol_type = other DNA
tgcaaggatcactcgccagatcacaagcgggagatcgatccggatc

SEQ ID NO: 162 - DNA, 46 bp, synthetic construct
  misc_feature 1..46: note = oligonucleotide primer
  source 1..46: mol_type = other DNA
tgcaaggatcactcgtccggtacgctatctgagatcgatccggatc

SEQ ID NO: 163 - DNA, 46 bp, synthetic construct
  misc_feature 1..46: note = oligonucleotide primer
  source 1..46: mol_type = other DNA
tgcaaggatcactcggatgatgagcctggagagatcgatccggatc

SEQ ID NO: 164 - DNA, 46 bp, synthetic construct
  misc_feature 1..46: note = oligonucleotide primer
  source 1..46: mol_type = other DNA
tgcaaggatcactcgttggctctagtactcgagatcgatccggatc

SEQ ID NO: 165 - DNA, 21 bp, synthetic construct
  misc_feature 1..21: note = oligonucleotide primer
  source 1..21: mol_type = other DNA
aatcgtagtccgcgcaatcag

SEQ ID NO: 166 - DNA, 21 bp, synthetic construct
  misc_feature 1..21: note = oligonucleotide primer
  source 1..21: mol_type = other DNA
acgatttgcaaggatcactcg

SEQ ID NO: 167 - DNA, 16 bp, synthetic construct
  misc_feature 1..16: note = spacer sequence
  source 1..16: mol_type = other DNA
gatccggatcgatctc

SEQ ID NO: 168 - DNA, 734 bp, synthetic construct
  misc_feature 1..734: note = extended recording tag construct
  source 1..734: mol_type = other DNA
aatcacggtacaagtcactcatccgtacgctatctgagaatcgtccagatccggcatgctagtatctggtgcagactacgattgttacagatcactcagatgatgagcacagaaaatcgtcgaatcttccatcaccatcgaacagttacgattaatgtagtccgcacaatcgaatgtctaacatgccgaatcccggacgtctccagcttctaaaccaacagtagtcgcacaaatcattgtacggtacaagatctaacgagagatgatcggatctgaccactttaaacactgattacgcagactacgattacgatttaagaatcctcgtccggtacaatcatagtccgcacaatcaaccgtgtcatgtgaagatcagatcgatctcgaatagcgtaccagacagtgatcttgcaaatcgtaatgtgtccgcgccaatcgatagccatgaatcccagtcgatctcccgcttgtgatctggcgatcgccttgtaccgtcgtacgatttgagatcacctcgttaactcaagctaaagatcgtccggatcgctttataaacatctgattgcgcggtacgattatcgtagtccgcacatatcgaacctgttgaagatccggatcgtctctccaggctcatcatccgagtgatccttgcaaataatcatgtccgcaccatcaggtgtctaacgcttgccggatccgaatcgatctctccaggctcatcatcgaagtgatgt

SEQ ID NO: 169 - protein, 10 aa, synthetic construct
  REGION 1..10: note = synthetic peptide
CPVQLWVDST

SEQ ID NO: 170 - protein, 10 aa, synthetic construct
  REGION 1..10: note = synthetic peptide
  VARIANT 1..10: note = Xaa = Any Amino Acid
CPXQXWXDXT

SEQ ID NO: 171 - protein, 8 aa, synthetic construct
  REGION 1..8: note = FLAG epitope peptide
DYKDDDDK

SEQ ID NO: 172 - protein, 14 aa, synthetic construct
  REGION 1..14: note = V5 epitope peptide
GKPIPNPLLGLDST

SEQ ID NO: 173 - protein, 10 aa, synthetic construct
  REGION 1..10: note = c-Myc epitope peptide
EQKLISEEDL

SEQ ID NO: 174 - protein, 9 aa, synthetic construct
  REGION 1..9: note = HA epitope peptide
YPYDVPDYA

SEQ ID NO: 175 - protein, 14 aa, synthetic construct
  REGION 1..14: note = V5 epitope peptide
GKPIPNPLLGLDST

SEQ ID NO: 176 - protein, 9 aa, synthetic construct
  REGION 1..9: note = StrepTag II peptide
NWSHPQFEK

SEQ ID NO: 177 - DNA, 36 bp, synthetic construct
  misc_feature 1..36: note = synthetic nucloetide
  misc_feature 11..22: note = compartment bar code n = A, C, T, or G
  misc_feature 23..27: note = unique molecular identifier n = A, T, C or G
  source 1..36: mol_type = other DNA
gcgcaatcagnnnnnnnnnnnnnnnnntgcaaggat

SEQ ID NO: 178-179 - skipped (2 entries)

SEQ ID NO: 180 - protein, 10 aa, synthetic construct
  REGION 1..10: note = butelase I peptide substrate
CGGSSGSNHV

SEQ ID NO: 181 - protein, 6 aa, synthetic construct
  REGION 1..6: note = Butelase I substrate
CGSNVH

SEQ ID NO: 182 - protein, 10 aa, synthetic construct
  REGION 1..10: note = cMyc tag
LDEESILKGE

SEQ ID NO: 183 - protein, 8 aa, synthetic construct
  REGION 1..8: note = HA tag
KDDDDKYD

SEQ ID NO: 184 - protein, 14 aa, synthetic construct
  REGION 1..14: note = epitope
VLPVRAGLWAEVDY

SEQ ID NO: 185 - DNA, 31 bp, synthetic construct
  source 1..31: mol_type = other DNA
  misc_feature 1..31: note = synthetic oligonucleotide
  misc_feature 1: note = 18-atom hexa-ethyleneglycol spacer
  misc_feature 31: note = three carbon (3C) spacer
cactcagtcctaacgcgtatacgcactcagt

SEQ ID NO: 186 - DNA, 32 bp, synthetic construct
  source 1..32: mol_type = other DNA
  misc_feature 1..32: note = synthetic oligonucleotide
  misc_feature 1: note = 18-atom hexa-ethyleneglycol spacer
  misc_feature 32: note = three carbon (3C) spacer
cactcagtcctaacgcgtatacgtcactcagt

SEQ ID NO: 187 - DNA, 32 bp, synthetic construct; identical to SEQ ID NO: 186
  source 1..32: mol_type = other DNA
  misc_feature 1..32: note = synthetic oligonucleotide
  misc_feature 1: note = five 18-atom hexa-ethyleneglycol spacer
  misc_feature 32: note = three carbon (3C) spacer

SEQ ID NO: 188 - DNA, 38 bp, synthetic construct
  source 1..38: mol_type = other DNA
  misc_feature 1..38: note = synthetic oligonucleotide
  misc_feature 1: note = 18-atom hexa-ethyleneglycol spacer
  misc_feature 38: note = three carbon (3C) spacer
cactcagtcctaacgcgtatacgggaatctcggcagtt